European Patent Application EP 4 809 830 A1, published September 23, 2026. Title: 2'-岩藻糖基乳糖在促进肠道发育、预防肠道损伤中的应用. Applicant: 澳优乳业（中国）有限公司. Application CN. The sequence listing filed with the application follows.

SEQUENCE LISTING (12 sequences)

SEQ ID NO: 1 - DNA, 24 bp, synthetic construct
  source 1..24: mol_type = other DNA
tattgccgaaatgtgctcaagggc

SEQ ID NO: 2 - DNA, 20 bp, synthetic construct
  source 1..20: mol_type = other DNA
ccacccagtacagcgtcaac

SEQ ID NO: 3 - DNA, 28 bp, synthetic construct
  source 1..28: mol_type = other DNA
tctttatgtgactcatctgtctcaccgg

SEQ ID NO: 4 - DNA, 17 bp, synthetic construct
  source 1..17: mol_type = other DNA
tataccgcgcgctccaa

SEQ ID NO: 5 - DNA, 20 bp, synthetic construct
  source 1..20: mol_type = other DNA
cataggcgatgagagattgt

SEQ ID NO: 6 - DNA, 22 bp, synthetic construct
  source 1..22: mol_type = other DNA
ggctacgatgtcagcattcctg

SEQ ID NO: 7 - DNA, 24 bp, synthetic construct
  source 1..24: mol_type = other DNA
atgacactctccacacccgatgta

SEQ ID NO: 8 - DNA, 20 bp, synthetic construct
  source 1..20: mol_type = other DNA
catggtgcttctgtcgctct

SEQ ID NO: 9 - DNA, 26 bp, synthetic construct
  source 1..26: mol_type = other DNA
ttgttggctaccagtttatccaaacg

SEQ ID NO: 10 - DNA, 21 bp, synthetic construct
  source 1..21: mol_type = other DNA
gccactcccggaagtaagact

SEQ ID NO: 11 - DNA, 20 bp, synthetic construct
  source 1..20: mol_type = other DNA
caagaattgtgtctgctgtc

SEQ ID NO: 12 - DNA, 22 bp, synthetic construct
  source 1..22: mol_type = other DNA
ggcttctaggtcctctctgtac